European Patent Application EP 4 541 888 A1, published April 23, 2025. Title: Allulose epimerase expression cassette and manufacturing method of allulose using the same. Applicant: DAESANG CORPORATION. The sequence listing filed with the application follows.

SEQUENCE LISTING (15 sequences)

SEQ ID NO: 1 - DNA, 200 bp, Corynebacterium glutamicum
  source 1..200: mol_type = genomic DNA
accctacttagctgccaattattccgggcttgtgacccgctacccgataaataggtcggctgaaaaatttcgttgcaatatcaacaaaaaggcctatcattgggaggtgtcgcaccaagtacttttgcgaagcgccatctgacggattttcaaaagatgtatatgctcggtgcggaaacctacgaaaggattttttaccc

SEQ ID NO: 2 - DNA, 885 bp, Flavonifractor plautii
  source 1..885: mol_type = genomic DNA
atgaacccgattggaatgcactacggcttctggagccacaactgggacgagattgcatacatacccctgatggagaagctggcctggctgggctttgacatctgcgaggtggcctccgccgagtggggctattacgacgacgccaggctgcgggagctgaaggcctgcgccgatcacaacggcctgggcatcacctattccatcggcctggaggccaaatacgacctggccagcgacgatccggcggtgcgggagaacggcatccgccatgtcacccgcatcctggagagcatgcccaaggtgggggcggccatcctcaacggcgtgtcctacgccgggtggcaggccctgcccgaccacggaatcaccctggacgagaagcgccgcaaggaggagcttgccctggagtccatgtcccggctcatgaaggtggcggaggactgcggcgtgctctactgctgcgaggtggtcaaccgcttcgagcagtacctgctcaacaccgccaaagagggcgtggagtttgtcaagcgcctgggcagtcccaacgcccgggtgctgctggataccttccacatgaacatcgaggaggacagcatggtggacgccattctggaggcgggcccctggctggggcatttccacgtgggggagaacaaccgccgccccgccggctccaccaaccgcctgccctggaaggacatggccgccgccctcaagcaggtgaactaccagggggccattgtgatggagcccttcgtgctcatggggggtaccattccctatgatatcaaggtctggcgggatctcagcggcggggccggggaggccgggctggacgagatggcgggccgggcctgccggttcctcaaggagctgaccgcgtaa

SEQ ID NO: 3 - protein, 294 aa, Flavonifractor plautii
MNPIGMHYGFWSHNWDEIAYIPLMEKLAWLGFDICEVASAEWGYYDDARLRELKACADHNGLGITYSIGLEAKYDLASDDPAVRENGIRHVTRILESMPKVGAAILNGVSYAGWQALPDHGITLDEKRRKEELALESMSRLMKVAEDCGVLYCCEVVNRFEQYLLNTAKEGVEFVKRLGSPNARVLLDTFHMNIEEDSMVDAILEAGPWLGHFHVGENNRRPAGSTNRLPWKDMAAALKQVNYQGAIVMEPFVLMGGTIPYDIKVWRDLSGGAGEAGLDEMAGRACRFLKELTA

SEQ ID NO: 4 - DNA, 795 bp, Escherichia coli
  source 1..795: mol_type = genomic DNA
atgattgaacaagatggattgcacgcaggttctccggccgcttgggtggagaggctattcggctatgactgggcacaacagacaatcggctgctctgatgccgccgtgttccggctgtcagcgcaggggcgcccggttctttttgtcaagaccgacctgtccggtgccctgaatgaactccaggacgaggcagcgcggctatcgtggctggccacgacgggcgttccttgcgcagctgtgctcgacgttgtcactgaagcgggaagggactggctgctattgggcgaagtgccggggcaggatctcctgtcatctcaccttgctcctgccgagaaagtatccatcatggctgatgcaatgcggcggctgcatacgcttgatccggctacctgcccattcgaccaccaagcgaaacatcgcatcgagcgagcacgtactcggatggaagccggtcttgtcgatcaggatgatctggacgaagagcatcaggggctcgcgccagccgaactgttcgccaggctcaaggcgcgcatgcccgacggcgaggatctcgtcgtgacacatggcgatgcctgcttgccgaatatcatggtggaaaatggccgcttttctggattcatcgactgtggccggctgggtgtggcggaccgctatcaggacatagcgttggctacccgtgatattgctgaagagcttggcggcgaatgggctgaccgcttcctcgtgctttacggtatcgccgctcccgattcgcagcgcatcgccttctatcgccttcttgacgagttcttctga

SEQ ID NO: 5 - DNA, 29 bp, synthetic construct
  source 1..29: mol_type = other DNA
agtcactgcagaccctacttagctgccaa

SEQ ID NO: 6 - DNA, 50 bp, synthetic construct
  source 1..50: mol_type = other DNA
aaacctacgaaaggattttttacccatgtgtcagatgaacccgattggaa

SEQ ID NO: 7 - DNA, 50 bp, synthetic construct
  source 1..50: mol_type = other DNA
ttccaatcgggttcatctgacacatgggtaaaaaatcctttcgtaggttt

SEQ ID NO: 8 - DNA, 30 bp, synthetic construct
  source 1..30: mol_type = other DNA
aattcggatccttacgcggtcagctccttg

SEQ ID NO: 9 - DNA, 200 bp, synthetic construct
  source 1..200: mol_type = other DNA
accctacttagctgccaattattccgggcttgtgacccgctacccgataaataggtcggctgaaaaatttcgttgcaatatcaacaaaaaggcctatcattgggaggtgtcgcaccaagtacttttgcgaagcgccatctgacggattttcaaaagatgtatatgctcggtgcggaaacctacgaaaggagattttaccc

SEQ ID NO: 10 - DNA, 200 bp, synthetic construct
  source 1..200: mol_type = other DNA
accctacttagctgccaattattccgggcttgtgacccgctacccgataaataggtcggctgaaaaatttcgttgcaatatcaacaaaaaggcctatcattgggaggtgtcgcaccaagtacttttgcgaagcgccatctgacggattttcaaaagatgtatatgctcggtgcggaaacctacgaaaggagtttttaccc

SEQ ID NO: 11 - DNA, 200 bp, synthetic construct
  source 1..200: mol_type = other DNA
accctacttagctgccaattattccgggcttgtgacccgctacccgataaataggtcggctgaaaaatttcgttgcaatatcaacaaaaaggcctatcattgggaggtgtcgcaccaagtacttttgcgaagcgccatctgacggattttcaaaagatgtatatgctcggtgcggaaacctacgaaaggagcttttaccc

SEQ ID NO: 12 - DNA, 885 bp, synthetic construct
  source 1..885: mol_type = other DNA
atgaacccgattggaatgcactacggcttctggagccacaactgggacgagattgcatacatacccctgatggagaagctggccaaactgggctttgacatctgcgaggtggcctccgccgagtggggctattacgacgacgccaggctgcgggagctgaaggcctgcgccgatcacaacggcctgggcatcacctattccatcggcctggaggccaaatacgacctggccagcgacgatccggcggtgcgggagaacggcatccgccatgtcacccgcatcctggagagcatgcccaaggtgggggcggccatcctcaacggcgtgtcctacgccgggtggcaggccctgcccgaccacggaatcaccctggacgagaagcgccgcaaggaggagcttgccctggagtccatgtcccggctcatgaaggtggcggaggactgcggcgtgctctactgctgcgaggtggtcaaccgcttcgagcagtacctgctcaacaccgccaaagagggcgtggagtttgtcaagcgcctgggcagtcccaacgcccgggtgctgctggataccttccacatgaacatcgaggaggacagcatggtggacgccattctggaggcgggcccctggctggggcatttccacgtgagcgagaacaaccgccgccccgccggctccaccaaccgcctgccctggaaggacattgccgccgccctcaagcaggtgaactaccagggggccattgtgatggagcccttcgtgctcatggggggtaccattccctatgatatcaaggtctggcgggatctcagcggcggggccggggaggccgggctggacgagatggcgggccgggcctgccggttcctcaaggagctgaccgcgtaa

SEQ ID NO: 13 - protein, 294 aa, synthetic construct
MNPIGMHYGFWSHNWDEIAYIPLMEKLAKLGFDICEVASAEWGYYDDARLRELKACADHNGLGITYSIGLEAKYDLASDDPAVRENGIRHVTRILESMPKVGAAILNGVSYAGWQALPDHGITLDEKRRKEELALESMSRLMKVAEDCGVLYCCEVVNRFEQYLLNTAKEGVEFVKRLGSPNARVLLDTFHMNIEEDSMVDAILEAGPWLGHFHVSENNRRPAGSTNRLPWKDIAAALKQVNYQGAIVMEPFVLMGGTIPYDIKVWRDLSGGAGEAGLDEMAGRACRFLKELTA

SEQ ID NO: 14 - DNA, 885 bp, synthetic construct
  source 1..885: mol_type = other DNA
atgaacccgattggaatgcactacggcttctggagccacaactgggacgagattgcatacatacccctgatggagaagctggccaaactgggctttgacatctgcgaggtggcctccgccgagtggggctattacgacgacgccaggctgcgggagctgaaggcctgcgccgatcacaacggcctgggcatcacctattccatcggcctggaggccaaatacgacctgagcagcgacgatccggcggtgcgggagaacggcatccgccatgtcacccgcatcctggagagcatgcccaaggtgggggcggccatcctcaacggcgtgtcctacgccgggtggcaggccctgcccgaccacggaatcaccctggacgagaagcgccgcaaggaggagcttgccctggagtccatgtcccggctcatgaaggtggcggaggactgcggcgtgctctactgctgcgaggtggtcaaccgcttcgagcagtacctgctcaacaccgccaaagagggcgtggagtttgtcaagcgcctgggcagtcccaacgcccgggtgctgctggataccttccacatgaacatcgaggaggacagcatggtggacgccattctggaggcgggcccctggctggggcatttccacgtgagcgagaacaaccgccgccccgccggctccaccaaccgcctgccctggaaggacattgccgccgccctcaagcaggtgaactaccagggggccattgtgatggagcccttcgtgctcatggggggtaccattccctatgatatcaaggtctggcgggatctcagcggcggggccggggaggccgggctggacgagatggcgggccgggcctgccggttcctcaaggagctgaccgcgtaa

SEQ ID NO: 15 - protein, 294 aa, synthetic construct
MNPIGMHYGFWSHNWDEIAYIPLMEKLAKLGFDICEVASAEWGYYDDARLRELKACADHNGLGITYSIGLEAKYDLSSDDPAVRENGIRHVTRILESMPKVGAAILNGVSYAGWQALPDHGITLDEKRRKEELALESMSRLMKVAEDCGVLYCCEVVNRFEQYLLNTAKEGVEFVKRLGSPNARVLLDTFHMNIEEDSMVDAILEAGPWLGHFHVSENNRRPAGSTNRLPWKDIAAALKQVNYQGAIVMEPFVLMGGTIPYDIKVWRDLSGGAGEAGLDEMAGRACRFLKELTA